European Patent Specification EP 3 720 883 B1, published April 19, 2023. Title: T-CELLS COMPRISING ANTI-CD38 AND ANTI-CD138 CHIMERIC ANTIGEN RECEPTORS AND USES THEREOF. Applicant: Aviv MedTech LTD. The sequence listing filed with the application follows.

SEQUENCE LISTING (39 sequences)

SEQ ID NO: 1 - protein, 6 aa, Artificial Sequence
  artificial sequence
QGINNY

SEQ ID NO: 2 - protein, 4 aa, Artificial Sequence
  artificial sequence
  SITE (4)..(4): X-any amino acid
YTSX

SEQ ID NO: 3 - protein, 9 aa, Artificial Sequence
  artificial sequence
QQYSKLPRT

SEQ ID NO: 4 - protein, 8 aa, Artificial Sequence
  artificial sequence
GYTFSNYW

SEQ ID NO: 5 - protein, 9 aa, Artificial Sequence
  artificial sequence
ILPGTGRTI

SEQ ID NO: 6 - protein, 15 aa, Artificial Sequence
  artificial sequence
ARRDYYGNFYYAMDY

SEQ ID NO: 7 - protein, 6 aa, Artificial Sequence
  artificial sequence
QSVSSY

SEQ ID NO: 8 - protein, 4 aa, Artificial Sequence
  artificial sequence
  site (4)..(4): X-any amino acid
DASX

SEQ ID NO: 9 - protein, 9 aa, Artificial Sequence
  artificial sequence
QQRSNWPPT

SEQ ID NO: 10 - protein, 8 aa, Artificial Sequence
  artificial sequence
GFTFNSFA

SEQ ID NO: 11 - protein, 9 aa, Artificial Sequence
  artificial sequence
ISGSGGGTY

SEQ ID NO: 12 - protein, 15 aa, Artificial Sequence
  artificial sequence
AKDKILWFGEPVFDY

SEQ ID NO: 13 - protein, 107 aa, Artificial Sequence
  artificial sequence
DIQMTQSTSSLSASLGDRVTISCSASQGINNYLNWYQQKPDGTVELLIYYTSTLQSGVPSRFSGSGSGTDYSLTISNLEPEDIGTYYCQQYSKLPRTFGGGTKLEIK

SEQ ID NO: 14 - protein, 122 aa, Artificial Sequence
  artificial sequence
QVQLQQSGSELMMPGASVKISCKATGYTFSNYWIEWVKQRPGHGLEWIGEILPGTGRTIYNEKFKGKATFTADISSNTVQMQLSSLTSEDSAVYYCARRDYYGNFYYAMDYWGQGTSVTVSS

SEQ ID NO: 15 - protein, 107 aa, Artificial Sequence [sequence omitted]

SEQ ID NO: 16 - protein, 122 aa, Artificial Sequence [sequence omitted]

SEQ ID NO: 17 - protein, 14 aa, Artificial Sequence
  artificial sequence
GSTSGSGKSSEGKG

SEQ ID NO: 18 - protein, 243 aa, Artificial Sequence
  artificial sequence
DIQMTQSTSSLSASLGDRVTISCSASQGINNYLNWYQQKPDGTVELLIYYTSTLQSGVPSRFSGSGSGTDYSLTISNLEPEDIGTYYCQQYSKLPRTFGGGTKLEIKGSTSGSGKSSEGKGQVQLQQSGSELMMPGASVKISCKATGYTFSNYWIEWVKQRPGHGLEWIGEILPGTGRTIYNEKFKGKATFTADISSNTVQMQLSSLTSEDSAVYYCARRDYYGNFYYAMDYWGQGTSVTVSS

SEQ ID NO: 19 - protein, 243 aa, Artificial Sequence
  artificial sequence
EIVLTQSPATLSLSPGERATLSCRASQSVSSYLAWYQQKPGQAPRLLIYDASNRATGIPARFSGSGSGTDFTLTISSLEPEDFAVYYCQQRSNWPPTFGQGTKVEIKGSTSGSGKSSEGKGEVQLLESGGGLVQPGGSLRLSCAVSGFTFNSFAMSWVRQAPGKGLEWVSAISGSGGGTYYADSVKGRFTISRDNSKNTLYLQMNSLRAEDTAVYFCAKDKILWFGEPVFDYWGQGTLVTVSS

SEQ ID NO: 20 - protein, 22 aa, Artificial Sequence
  artificial sequence
MDFQVQIFSFLLISASVIMSRG

SEQ ID NO: 21 - protein, 772 aa, Artificial Sequence
  artificial sequence
MDFQVQIFSFLLISASVIMSRGDIQMTQSTSSLSASLGDRVTISCSASQGINNYLNWYQQKPDGTVELLIYYTSTLQSGVPSRFSGSGSGTDYSLTISNLEPEDIGTYYCQQYSKLPRTFGGGTKLEIKGSTSGSGKSSEGKGQVQLQQSGSELMMPGASVKISCKATGYTFSNYWIEWVKQRPGHGLEWIGEILPGTGRTIYNEKFKGKATFTADISSNTVQMQLSSLTSEDSAVYYCARRDYYGNFYYAMDYWGQGTSVTVSSAAAKGKHLCPSPLFPGPSKPFWVLVVVGGVLACYSLLVTVAFIIFWVRSKRSRLLHSDYMNMTPRRPGPTRKHYQPYAPPRDFAAYRSGSGEGRGSLLTCGDVEENPGPYVMDFQVQIFSFLLISASVIMSRGEIVLTQSPATLSLSPGERATLSCRASQSVSSYLAWYQQKPGQAPRLLIYDASNRATGIPARFSGSGSGTDFTLTISSLEPEDFAVYYCQQRSNWPPTFGQGTKVEIKGSTSGSGKSSEGKGEVQLLESGGGLVQPGGSLRLSCAVSGFTFNSFAMSWVRQAPGKGLEWVSAISGSGGGTYYADSVKGRFTISRDNSKNTLYLQMNSLRAEDTAVYFCAKDKILWFGEPVFDYWGQGTLVTVSSLSNSIMYFSHFVPVFLPAKPTTTPAPRPPTPAPTIASQPLSLRPEACRPAAGGAVHTRGLDFACDIYIWAPLAGTCGVLLLSLVITLYCNHRSQVRKAAITSYEKSDGVYTGLSTRNQETYETLKHEKPPQ

SEQ ID NO: 22 - protein, 40 aa, Artificial Sequence
  artificial sequence
SKRSRLLHSDYMNMTPRRPGPTRKHYQPYAPPRDFAAYRS

SEQ ID NO: 23 - protein, 40 aa, Artificial Sequence
  artificial sequence
RSQVRKAAITSYEKSDGVYTGLSTRNQETYETLKHEKPPQ

SEQ ID NO: 24 - protein, 353 aa, Artificial Sequence
  artificial sequence
MDFQVQIFSFLLISASVIMSRGDIQMTQSTSSLSASLGDRVTISCSASQGINNYLNWYQQKPDGTVELLIYYTSTLQSGVPSRFSGSGSGTDYSLTISNLEPEDIGTYYCQQYSKLPRTFGGGTKLEIKGSTSGSGKSSEGKGQVQLQQSGSELMMPGASVKISCKATGYTFSNYWIEWVKQRPGHGLEWIGEILPGTGRTIYNEKFKGKATFTADISSNTVQMQLSSLTSEDSAVYYCARRDYYGNFYYAMDYWGQGTSVTVSSAAAKGKHLCPSPLFPGPSKPFWVLVVVGGVLACYSLLVTVAFIIFWVRSKRSRLLHSDYMNMTPRRPGPTRKHYQPYAPPRDFAAYRS

SEQ ID NO: 25 - protein, 398 aa, Artificial Sequence
  artificial sequence
YVMDFQVQIFSFLLISASVIMSRGEIVLTQSPATLSLSPGERATLSCRASQSVSSYLAWYQQKPGQAPRLLIYDASNRATGIPARFSGSGSGTDFTLTISSLEPEDFAVYYCQQRSNWPPTFGQGTKVEIKGSTSGSGKSSEGKGEVQLLESGGGLVQPGGSLRLSCAVSGFTFNSFAMSWVRQAPGKGLEWVSAISGSGGGTYYADSVKGRFTISRDNSKNTLYLQMNSLRAEDTAVYFCAKDKILWFGEPVFDYWGQGTLVTVSSLSNSIMYFSHFVPVFLPAKPTTTPAPRPPTPAPTIASQPLSLRPEACRPAAGGAVHTRGLDFACDIYIWAPLAGTCGVLLLSLVITLYCNHRSQVRKAAITSYEKSDGVYTGLSTRNQETYETLKHEKPPQ

SEQ ID NO: 26 - protein, 20 aa, Artificial Sequence
  artificial sequence
GSGEGRGSLLTCGDVEENPG

SEQ ID NO: 27 - DNA, 63 bp, Artificial Sequence
  artificial sequence
ggctccggagagggcagaggaagtcttctaacatgcggtgacgtggaggagaatcccggccct

SEQ ID NO: 28 - DNA, 729 bp, Artificial Sequence
  artificial sequence
gatatccagatgacacagagtacatcctccctgtctgcctctctgggagacagagtcaccatcagttgcagtgcaagtcagggcattaacaattatttaaactggtatcagcagaaaccagatggaactgttgaactcctgatctattacacatcaactttacagtcaggagtcccatcaaggttcagtggcagtgggtctgggacagattattctctcaccatcagcaacctggaacctgaagatattggcacttactattgtcagcagtatagtaagcttcctcggacgttcggtggaggcaccaagctggaaatcaaagggtcgacttccggtagcggcaaatcctctgaaggcaaaggtcaggttcagctgcagcagtctggatctgagctgatgatgcctggggcctcagtgaagatatcctgcaaggctactggctacacattcagtaactactggatagagtgggtaaagcagaggcctggacatggccttgagtggattggagagattttacctggaactggtagaactatctacaatgagaagttcaagggcaaggccacattcactgcagatatatcctccaacacagtccaaatgcaactcagcagcctgacatctgaggactctgccgtctattactgtgcaagaagggactattatggtaacttttactatgctatggactactggggtcaagggacctcagtcaccgtctcctca

SEQ ID NO: 29 - DNA, 729 bp, Artificial Sequence
  artificial sequence
gaaattgtgttgacgcagtctccagccaccctgtctttgtctccaggggaaagagccaccctctcctgcagggccagtcagagtgttagcagctacttagcctggtaccaacagaaacctggccaggctcccaggctcctcatctatgatgcatccaacagggccactggcattccagccaggttcagtggcagtgggtctgggacagacttcactctcaccatcagcagcctagagcctgaagattttgcagtttattactgtcagcagcgtagcaactggcctccgacgttcggccaagggaccaaggtggaaatcaaagggtcgacttccggtagcggcaaatcctctgaaggcaaaggtgaggtgcagctgttggagtctgggggaggcttggtacagcctggggggtccctgagactctcctgtgcagtctctggattcacctttaacagctttgccatgagctgggtccgccaggctccagggaaggggctggagtgggtctcagctattagtggtagtggtggtggcacatactacgcagactccgtgaagggccggttcaccatctccagagacaattccaagaacacgctgtatctgcaaatgaacagcctgagagccgaggacacggccgtatatttctgtgcgaaagataagattttatggtttggggagccggtcttcgactactggggccagggaaccctggtcaccgtctcctca

SEQ ID NO: 30 - DNA, 120 bp, Artificial Sequence
  artificial sequence
agtaagaggagcaggctcctgcacagtgactacatgaacatgactccccgccgccccgggcccacccgcaagcattaccagccctatgccccaccacgcgacttcgcagcctatagatct

SEQ ID NO: 31 - DNA, 130 bp, Artificial Sequence
  artificial sequence
agatctcaagtgcgaaaggcagctataaccagctatgagaaatcagatggtgtttacacgggcctgagcaccaggaaccaggagacttacgagactctgaagcatgagaaaccaccacagtagactcgag

SEQ ID NO: 32 - DNA, 1059 bp, Artificial Sequence
  artificial sequence
atggattttcaggtgcagattttcagcttcctgctaatcagtgcctcagtcataatgtccagaggagatatccagatgacacagagtacatcctccctgtctgcctctctgggagacagagtcaccatcagttgcagtgcaagtcagggcattaacaattatttaaactggtatcagcagaaaccagatggaactgttgaactcctgatctattacacatcaactttacagtcaggagtcccatcaaggttcagtggcagtgggtctgggacagattattctctcaccatcagcaacctggaacctgaagatattggcacttactattgtcagcagtatagtaagcttcctcggacgttcggtggaggcaccaagctggaaatcaaagggtcgacttccggtagcggcaaatcctctgaaggcaaaggtcaggttcagctgcagcagtctggatctgagctgatgatgcctggggcctcagtgaagatatcctgcaaggctactggctacacattcagtaactactggatagagtgggtaaagcagaggcctggacatggccttgagtggattggagagattttacctggaactggtagaactatctacaatgagaagttcaagggcaaggccacattcactgcagatatatcctccaacacagtccaaatgcaactcagcagcctgacatctgaggactctgccgtctattactgtgcaagaagggactattatggtaacttttactatgctatggactactggggtcaagggacctcagtcaccgtctcctcagcggccgcaaaagggaaacacctttgtccaagtcccctatttcccggaccttctaagcccttttgggtgctggtggtggttggtggagtcctggcttgctatagcttgctagtaacagtggcctttattattttctgggtgaggagtaagaggagcaggctcctgcacagtgactacatgaacatgactccccgccgccccgggcccacccgcaagcattaccagccctatgccccaccacgcgacttcgcagcctatagatct

SEQ ID NO: 33 - DNA, 1198 bp, Artificial Sequence
  artificial sequence
atggattttcaggtgcagattttcagcttcctgctaatcagtgcctcagtcataatgtccagaggagaaattgtgttgacgcagtctccagccaccctgtctttgtctccaggggaaagagccaccctctcctgcagggccagtcagagtgttagcagctacttagcctggtaccaacagaaacctggccaggctcccaggctcctcatctatgatgcatccaacagggccactggcattccagccaggttcagtggcagtgggtctgggacagacttcactctcaccatcagcagcctagagcctgaagattttgcagtttattactgtcagcagcgtagcaactggcctccgacgttcggccaagggaccaaggtggaaatcaaagggtcgacttccggtagcggcaaatcctctgaaggcaaaggtgaggtgcagctgttggagtctgggggaggcttggtacagcctggggggtccctgagactctcctgtgcagtctctggattcacctttaacagctttgccatgagctgggtccgccaggctccagggaaggggctggagtgggtctcagctattagtggtagtggtggtggcacatactacgcagactccgtgaagggccggttcaccatctccagagacaattccaagaacacgctgtatctgcaaatgaacagcctgagagccgaggacacggccgtatatttctgtgcgaaagataagattttatggtttggggagccggtcttcgactactggggccagggaaccctggtcaccgtctcctcactgagcaactccatcatgtacttcagccacttcgtgccggtcttcctgccagcgaagcccaccacgacgccagcgccgcgaccaccaacaccggcgcccaccatcgcgtcgcagcccctgtccctgcgcccagaggcgtgccggccagcggcggggggcgcagtgcacacgagggggctggacttcgcctgtgatatctacatctgggcgcccttggccgggacttgtggggtccttctcctgtcactggttatcaccctttactgcaaccacagatctcaagtgcgaaaggcagctataaccagctatgagaaatcagatggtgtttacacgggcctgagcaccaggaaccaggagacttacgagactctgaagcatgagaaaccaccacagtagactcgag

SEQ ID NO: 34 - DNA, 2319 bp, artificial sequenc
  artificial sequence
atggattttcaggtgcagattttcagcttcctgctaatcagtgcctcagtcataatgtccagaggagatatccagatgacacagagtacatcctccctgtctgcctctctgggagacagagtcaccatcagttgcagtgcaagtcagggcattaacaattatttaaactggtatcagcagaaaccagatggaactgttgaactcctgatctattacacatcaactttacagtcaggagtcccatcaaggttcagtggcagtgggtctgggacagattattctctcaccatcagcaacctggaacctgaagatattggcacttactattgtcagcagtatagtaagcttcctcggacgttcggtggaggcaccaagctggaaatcaaagggtcgacttccggtagcggcaaatcctctgaaggcaaaggtcaggttcagctgcagcagtctggatctgagctgatgatgcctggggcctcagtgaagatatcctgcaaggctactggctacacattcagtaactactggatagagtgggtaaagcagaggcctggacatggccttgagtggattggagagattttacctggaactggtagaactatctacaatgagaagttcaagggcaaggccacattcactgcagatatatcctccaacacagtccaaatgcaactcagcagcctgacatctgaggactctgccgtctattactgtgcaagaagggactattatggtaacttttactatgctatggactactggggtcaagggacctcagtcaccgtctcctcagcggccgcaaaagggaaacacctttgtccaagtcccctatttcccggaccttctaagcccttttgggtgctggtggtggttggtggagtcctggcttgctatagcttgctagtaacagtggcctttattattttctgggtgaggagtaagaggagcaggctcctgcacagtgactacatgaacatgactccccgccgccccgggcccacccgcaagcattaccagccctatgccccaccacgcgacttcgcagcctatagatctggctccggagagggcagaggaagtcttctaacatgcggtgacgtggaggagaatcccggcccttacgtaatggattttcaggtgcagattttcagcttcctgctaatcagtgcctcagtcataatgtccagaggagaaattgtgttgacgcagtctccagccaccctgtctttgtctccaggggaaagagccaccctctcctgcagggccagtcagagtgttagcagctacttagcctggtaccaacagaaacctggccaggctcccaggctcctcatctatgatgcatccaacagggccactggcattccagccaggttcagtggcagtgggtctgggacagacttcactctcaccatcagcagcctagagcctgaagattttgcagtttattactgtcagcagcgtagcaactggcctccgacgttcggccaagggaccaaggtggaaatcaaagggtcgacttccggtagcggcaaatcctctgaaggcaaaggtgaggtgcagctgttggagtctgggggaggcttggtacagcctggggggtccctgagactctcctgtgcagtctctggattcacctttaacagctttgccatgagctgggtccgccaggctccagggaaggggctggagtgggtctcagctattagtggtagtggtggtggcacatactacgcagactccgtgaagggccggttcaccatctccagagacaattccaagaacacgctgtatctgcaaatgaacagcctgagagccgaggacacggccgtatatttctgtgcgaaagataagattttatggtttggggagccggtcttcgactactggggccagggaaccctggtcaccgtctcctcactgagcaactccatcatgtacttcagccacttcgtgccggtcttcctgccagcgaagcccaccacgacgccagcgccgcgaccaccaacaccggcgcccaccatcgcgtcgcagcccctgtccctgcgcccagaggcgtgccggccagcggcggggggcgcagtgcacacgagggggctggacttcgcctgtgatatctacatctgggcgcccttggccgggacttgtggggtccttctcctgtcactggttatcaccctttactgcaaccacagatctcaagtgcgaaaggcagctataaccagctatgagaaatcagatggtgtttacacgggcctgagcaccaggaaccaggagacttacgagactctgaagcatgagaaaccaccacagtag

SEQ ID NO: 35 - protein, 45 aa, Artificial Sequence
  artificial sequence
KGKHLCPSPLFPGPSKPFWVLVVVGGVLACYSLLVTVAFIIFWVR

SEQ ID NO: 36 - protein, 91 aa, Artificial Sequence
  artificial sequence
LSNSIMYFSHFVPVFLPAKPTTTPAPRPPTPAPTIASQPLSLRPEACRPAAGGAVHTRGLDFACDIYIWAPLAGTCGVLLLSLVITLYCNH

SEQ ID NO: 37 - DNA, 134 bp, artificial sequence
  artificial sequence
aaagggaaacacctttgtccaagtcccctatttcccggaccttctaagcccttttgggtgctggtggtggttggtggagtcctggcttgctatagcttgctagtaacagtggcctttattattttctgggtgag

SEQ ID NO: 38 - DNA, 273 bp, Artificial Sequence
  artificial sequence
ctgagcaactccatcatgtacttcagccacttcgtgccggtcttcctgccagcgaagcccaccacgacgccagcgccgcgaccaccaacaccggcgcccaccatcgcgtcgcagcccctgtccctgcgcccagaggcgtgccggccagcggcggggggcgcagtgcacacgagggggctggacttcgcctgtgatatctacatctgggcgcccttggccgggacttgtggggtccttctcctgtcactggttatcaccctttactgcaaccac

SEQ ID NO: 39 - DNA, 66 bp, Artificial Sequence
  artificial sequence
atggattttcaggtgcagattttcagcttcctgctaatcagtgcctcagtcataatgtccagagga